European Patent Application EP 4 512 821 A1, published February 26, 2025. Title: Novel gluconate repressor variant and a method for producing L-arginine using the same. Applicant: CJ CheilJedang Corporation. The sequence listing filed with the application follows.

SEQUENCE LISTING (36 sequences)

SEQ ID NO: 1 - protein, 250 aa, unidentified
  REGION 1..250: note = gluconate repressor
MPPANESPMTNPLGSAPTPAKPLLDSVLDELGQDIISGKVAVGDTFKLMDIGERFGISRTVAREAMRALEQLGLVASSRRIGITVLPQEEWAVFDKSIIRWRLNDEGQREGQLQSLTELRIAIEPIAARSVALHASTAELEKIRALATEMRQLGESGQGASQRFLEADVTFHELILRYCHNEMFAALIPSISAVLVGRTELGLQPDLPAHEALDNHDKLADALLNRDADAAETASRNILNEVRSALGTLN

SEQ ID NO: 2 - DNA, 753 bp, unidentified
  misc_feature 1..753: note = gluconate repressor
  source 1..753: mol_type = genomic DNA
atgcccccagcaaacgaaagtcctatgactaatccattaggttctgcccccaccccagccaagccacttcttgacagtgttcttgatgagctcggtcaagatatcatcagtggcaaggttgctgtcggagataccttcaagctgatggacatcggcgagcgttttggtatttcccgcacagtggcacgcgaagcaatgcgcgctttggagcagctcggtcttgtcgcttcttcacgtcgcattggcattactgttttgccacaggaagagtgggctgtttttgataagtccatcattcgctggcgtctcaatgacgaaggtcagcgtgaaggccagcttcagtctcttaccgagcttcgtattgctattgaaccgattgccgcgcgcagcgttgctcttcacgcgtcaaccgccgagctcgagaaaatccgcgcgctggcaacagagatgcgtcagttgggtgaatctggtcagggtgcgtcccagcgcttcctcgaagcggacgtcaccttccacgagctcatcttgcgttattgccacaatgagatgttcgctgcactgattccgtcgattagcgcggttcttgtcggccgcaccgagctcggcctgcagcctgatctgccggcgcacgaggcgctagacaaccacgataagcttgccgacgccctccttaaccgcgacgccgacgccgcagaaactgcgtcccgaaacatcctcaatgaggtgcgcagcgcgctgggcacgctgaactaa

SEQ ID NO: 3 - DNA, 34 bp, synthetic construct
  misc_feature 1..34: note = primer
  source 1..34: mol_type = other DNA
tcggtacccggggatccaagcaaccgtcggcgag

SEQ ID NO: 4 - DNA, 34 bp, synthetic construct
  misc_feature 1..34: note = primer
  source 1..34: mol_type = other DNA
tgcaggtcgactctagatttcgggacgcagtttc

SEQ ID NO: 5 - DNA, 34 bp, synthetic construct
  misc_feature 1..34: note = primer
  source 1..34: mol_type = other DNA
agcaaccttgccactgttgatatcttgaccgagc

SEQ ID NO: 6 - DNA, 35 bp, synthetic construct
  misc_feature 1..35: note = primer
  source 1..35: mol_type = other DNA
acagtggcaaggttgctgtcggagataccttcaag

SEQ ID NO: 7 - DNA, 33 bp, synthetic construct
  misc_feature 1..33: note = primer
  source 1..33: mol_type = other DNA
tcgcgtgccactgtggcggaaataccaaaacgc

SEQ ID NO: 8 - DNA, 33 bp, synthetic construct
  misc_feature 1..33: note = primer
  source 1..33: mol_type = other DNA
gccacagtggcacgcgaagcaatgcgcgctttg

SEQ ID NO: 9 - DNA, 35 bp, synthetic construct
  misc_feature 1..35: note = primer
  source 1..35: mol_type = other DNA
gcttcgcgtgccactaggcgggaaataccaaaacg

SEQ ID NO: 10 - DNA, 35 bp, synthetic construct
  misc_feature 1..35: note = primer
  source 1..35: mol_type = other DNA
ctagtggcacgcgaagcaatgcgcgctttggagca

SEQ ID NO: 11 - DNA, 31 bp, synthetic construct
  misc_feature 1..31: note = primer
  source 1..31: mol_type = other DNA
gcgcgcattgcttcggctgccactgtgcggg

SEQ ID NO: 12 - DNA, 34 bp, synthetic construct
  misc_feature 1..34: note = primer
  source 1..34: mol_type = other DNA
gccgaagcaatgcgcgctttggagcagctcggtc

SEQ ID NO: 13 - DNA, 34 bp, synthetic construct
  misc_feature 1..34: note = primer
  source 1..34: mol_type = other DNA
cgagctgcttcaaagcgcgcattgcttcgcgtgc

SEQ ID NO: 14 - DNA, 35 bp, synthetic construct
  misc_feature 1..35: note = primer
  source 1..35: mol_type = other DNA
cgctttgaagcagctcggtcttgtcgcttcttcac

SEQ ID NO: 15 - DNA, 35 bp, synthetic construct
  misc_feature 1..35: note = primer
  source 1..35: mol_type = other DNA
gtaatgccaatgcgagctgaagaagcgacaagacc

SEQ ID NO: 16 - DNA, 34 bp, synthetic construct
  misc_feature 1..34: note = primer
  source 1..34: mol_type = other DNA
gctcgcattggcattactgttttgccacaggaag

SEQ ID NO: 17 - DNA, 33 bp, synthetic construct
  misc_feature 1..33: note = primer
  source 1..33: mol_type = other DNA
gacttatcaaaaacaagccactcttcctgtggc

SEQ ID NO: 18 - DNA, 34 bp, synthetic construct
  misc_feature 1..34: note = primer
  source 1..34: mol_type = other DNA
cttgtttttgataagtccatcattcgctggcgtc

SEQ ID NO: 19 - DNA, 36 bp, synthetic construct
  misc_feature 1..36: note = primer
  source 1..36: mol_type = other DNA
tcggtacccggggatccagcaggccttaagggtaag

SEQ ID NO: 20 - DNA, 34 bp, synthetic construct
  misc_feature 1..34: note = primer
  source 1..34: mol_type = other DNA
aggggcgctgtcttacctcggctggtgggccagc

SEQ ID NO: 21 - DNA, 36 bp, synthetic construct
  misc_feature 1..36: note = primer
  source 1..36: mol_type = other DNA
ggtaagacagcgcccctagttcaaggcttgttaatc

SEQ ID NO: 22 - DNA, 37 bp, synthetic construct
  misc_feature 1..37: note = primer
  source 1..37: mol_type = other DNA
tgcaggtcgactctagaaccgttgaactgcttgccag

SEQ ID NO: 23 - protein, 250 aa, synthetic construct
  REGION 1..250: note = gluconate repressor variant
MPPANESPMTNPLGSAPTPAKPLLDSVLDELGQDINSGKVAVGDTFKLMDIGERFGISRTVAREAMRALEQLGLVASSRRIGITVLPQEEWAVFDKSIIRWRLNDEGQREGQLQSLTELRIAIEPIAARSVALHASTAELEKIRALATEMRQLGESGQGASQRFLEADVTFHELILRYCHNEMFAALIPSISAVLVGRTELGLQPDLPAHEALDNHDKLADALLNRDADAAETASRNILNEVRSALGTLN

SEQ ID NO: 24 - protein, 250 aa, synthetic construct
  REGION 1..250: note = gluconate repressor variant
MPPANESPMTNPLGSAPTPAKPLLDSVLDELGQDIISGKVAVGDTFKLMDIGERFGISATVAREAMRALEQLGLVASSRRIGITVLPQEEWAVFDKSIIRWRLNDEGQREGQLQSLTELRIAIEPIAARSVALHASTAELEKIRALATEMRQLGESGQGASQRFLEADVTFHELILRYCHNEMFAALIPSISAVLVGRTELGLQPDLPAHEALDNHDKLADALLNRDADAAETASRNILNEVRSALGTLN

SEQ ID NO: 25 - protein, 250 aa, synthetic construct
  REGION 1..250: note = gluconate repressor variant
MPPANESPMTNPLGSAPTPAKPLLDSVLDELGQDIISGKVAVGDTFKLMDIGERFGISRLVAREAMRALEQLGLVASSRRIGITVLPQEEWAVFDKSIIRWRLNDEGQREGQLQSLTELRIAIEPIAARSVALHASTAELEKIRALATEMRQLGESGQGASQRFLEADVTFHELILRYCHNEMFAALIPSISAVLVGRTELGLQPDLPAHEALDNHDKLADALLNRDADAAETASRNILNEVRSALGTLN

SEQ ID NO: 26 - protein, 250 aa, synthetic construct
  REGION 1..250: note = gluconate repressor variant
MPPANESPMTNPLGSAPTPAKPLLDSVLDELGQDIISGKVAVGDTFKLMDIGERFGISRTVAAEAMRALEQLGLVASSRRIGITVLPQEEWAVFDKSIIRWRLNDEGQREGQLQSLTELRIAIEPIAARSVALHASTAELEKIRALATEMRQLGESGQGASQRFLEADVTFHELILRYCHNEMFAALIPSISAVLVGRTELGLQPDLPAHEALDNHDKLADALLNRDADAAETASRNILNEVRSALGTLN

SEQ ID NO: 27 - protein, 250 aa, synthetic construct
  REGION 1..250: note = gluconate repressor variant
MPPANESPMTNPLGSAPTPAKPLLDSVLDELGQDIISGKVAVGDTFKLMDIGERFGISRTVAREAMRALKQLGLVASSRRIGITVLPQEEWAVFDKSIIRWRLNDEGQREGQLQSLTELRIAIEPIAARSVALHASTAELEKIRALATEMRQLGESGQGASQRFLEADVTFHELILRYCHNEMFAALIPSISAVLVGRTELGLQPDLPAHEALDNHDKLADALLNRDADAAETASRNILNEVRSALGTLN

SEQ ID NO: 28 - protein, 250 aa, synthetic construct
  REGION 1..250: note = gluconate repressor variant
MPPANESPMTNPLGSAPTPAKPLLDSVLDELGQDIISGKVAVGDTFKLMDIGERFGISRTVAREAMRALEQLGLVASSARIGITVLPQEEWAVFDKSIIRWRLNDEGQREGQLQSLTELRIAIEPIAARSVALHASTAELEKIRALATEMRQLGESGQGASQRFLEADVTFHELILRYCHNEMFAALIPSISAVLVGRTELGLQPDLPAHEALDNHDKLADALLNRDADAAETASRNILNEVRSALGTLN

SEQ ID NO: 29 - protein, 250 aa, synthetic construct
  REGION 1..250: note = gluconate repressor variant
MPPANESPMTNPLGSAPTPAKPLLDSVLDELGQDIISGKVAVGDTFKLMDIGERFGISRTVAREAMRALEQLGLVASSRRIGITVLPQEEWLVFDKSIIRWRLNDEGQREGQLQSLTELRIAIEPIAARSVALHASTAELEKIRALATEMRQLGESGQGASQRFLEADVTFHELILRYCHNEMFAALIPSISAVLVGRTELGLQPDLPAHEALDNHDKLADALLNRDADAAETASRNILNEVRSALGTLN

SEQ ID NO: 30 - DNA, 753 bp, synthetic construct
  misc_feature 1..753: note = gluconate repressor variant
  source 1..753: mol_type = other DNA
atgcccccagcaaacgaaagtcctatgactaatccattaggttctgcccccaccccagccaagccacttcttgacagtgttcttgatgagctcggtcaagatatcaacagtggcaaggttgctgtcggagataccttcaagctgatggacatcggcgagcgttttggtatttcccgcacagtggcacgcgaagcaatgcgcgctttggagcagctcggtcttgtcgcttcttcacgtcgcattggcattactgttttgccacaggaagagtgggctgtttttgataagtccatcattcgctggcgtctcaatgacgaaggtcagcgtgaaggccagcttcagtctcttaccgagcttcgtattgctattgaaccgattgccgcgcgcagcgttgctcttcacgcgtcaaccgccgagctcgagaaaatccgcgcgctggcaacagagatgcgtcagttgggtgaatctggtcagggtgcgtcccagcgcttcctcgaagcggacgtcaccttccacgagctcatcttgcgttattgccacaatgagatgttcgctgcactgattccgtcgattagcgcggttcttgtcggccgcaccgagctcggcctgcagcctgatctgccggcgcacgaggcgctagacaaccacgataagcttgccgacgccctccttaaccgcgacgccgacgccgcagaaactgcgtcccgaaacatcctcaatgaggtgcgcagcgcgctgggcacgctgaactaa

SEQ ID NO: 31 - DNA, 753 bp, synthetic construct
  misc_feature 1..753: note = gluconate repressor variant
  source 1..753: mol_type = other DNA
atgcccccagcaaacgaaagtcctatgactaatccattaggttctgcccccaccccagccaagccacttcttgacagtgttcttgatgagctcggtcaagatatcatcagtggcaaggttgctgtcggagataccttcaagctgatggacatcggcgagcgttttggtatttccgccacagtggcacgcgaagcaatgcgcgctttggagcagctcggtcttgtcgcttcttcacgtcgcattggcattactgttttgccacaggaagagtgggctgtttttgataagtccatcattcgctggcgtctcaatgacgaaggtcagcgtgaaggccagcttcagtctcttaccgagcttcgtattgctattgaaccgattgccgcgcgcagcgttgctcttcacgcgtcaaccgccgagctcgagaaaatccgcgcgctggcaacagagatgcgtcagttgggtgaatctggtcagggtgcgtcccagcgcttcctcgaagcggacgtcaccttccacgagctcatcttgcgttattgccacaatgagatgttcgctgcactgattccgtcgattagcgcggttcttgtcggccgcaccgagctcggcctgcagcctgatctgccggcgcacgaggcgctagacaaccacgataagcttgccgacgccctccttaaccgcgacgccgacgccgcagaaactgcgtcccgaaacatcctcaatgaggtgcgcagcgcgctgggcacgctgaactaa

SEQ ID NO: 32 - DNA, 753 bp, synthetic construct
  misc_feature 1..753: note = gluconate repressor variant
  source 1..753: mol_type = other DNA
atgcccccagcaaacgaaagtcctatgactaatccattaggttctgcccccaccccagccaagccacttcttgacagtgttcttgatgagctcggtcaagatatcatcagtggcaaggttgctgtcggagataccttcaagctgatggacatcggcgagcgttttggtatttcccgcctagtggcacgcgaagcaatgcgcgctttggagcagctcggtcttgtcgcttcttcacgtcgcattggcattactgttttgccacaggaagagtgggctgtttttgataagtccatcattcgctggcgtctcaatgacgaaggtcagcgtgaaggccagcttcagtctcttaccgagcttcgtattgctattgaaccgattgccgcgcgcagcgttgctcttcacgcgtcaaccgccgagctcgagaaaatccgcgcgctggcaacagagatgcgtcagttgggtgaatctggtcagggtgcgtcccagcgcttcctcgaagcggacgtcaccttccacgagctcatcttgcgttattgccacaatgagatgttcgctgcactgattccgtcgattagcgcggttcttgtcggccgcaccgagctcggcctgcagcctgatctgccggcgcacgaggcgctagacaaccacgataagcttgccgacgccctccttaaccgcgacgccgacgccgcagaaactgcgtcccgaaacatcctcaatgaggtgcgcagcgcgctgggcacgctgaactaa

SEQ ID NO: 33 - DNA, 753 bp, synthetic construct
  misc_feature 1..753: note = gluconate repressor variant
  source 1..753: mol_type = other DNA
atgcccccagcaaacgaaagtcctatgactaatccattaggttctgcccccaccccagccaagccacttcttgacagtgttcttgatgagctcggtcaagatatcatcagtggcaaggttgctgtcggagataccttcaagctgatggacatcggcgagcgttttggtatttcccgcacagtggcagccgaagcaatgcgcgctttggagcagctcggtcttgtcgcttcttcacgtcgcattggcattactgttttgccacaggaagagtgggctgtttttgataagtccatcattcgctggcgtctcaatgacgaaggtcagcgtgaaggccagcttcagtctcttaccgagcttcgtattgctattgaaccgattgccgcgcgcagcgttgctcttcacgcgtcaaccgccgagctcgagaaaatccgcgcgctggcaacagagatgcgtcagttgggtgaatctggtcagggtgcgtcccagcgcttcctcgaagcggacgtcaccttccacgagctcatcttgcgttattgccacaatgagatgttcgctgcactgattccgtcgattagcgcggttcttgtcggccgcaccgagctcggcctgcagcctgatctgccggcgcacgaggcgctagacaaccacgataagcttgccgacgccctccttaaccgcgacgccgacgccgcagaaactgcgtcccgaaacatcctcaatgaggtgcgcagcgcgctgggcacgctgaactaa

SEQ ID NO: 34 - DNA, 753 bp, synthetic construct
  misc_feature 1..753: note = gluconate repressor variant
  source 1..753: mol_type = other DNA
atgcccccagcaaacgaaagtcctatgactaatccattaggttctgcccccaccccagccaagccacttcttgacagtgttcttgatgagctcggtcaagatatcatcagtggcaaggttgctgtcggagataccttcaagctgatggacatcggcgagcgttttggtatttcccgcacagtggcacgcgaagcaatgcgcgctttgaagcagctcggtcttgtcgcttcttcacgtcgcattggcattactgttttgccacaggaagagtgggctgtttttgataagtccatcattcgctggcgtctcaatgacgaaggtcagcgtgaaggccagcttcagtctcttaccgagcttcgtattgctattgaaccgattgccgcgcgcagcgttgctcttcacgcgtcaaccgccgagctcgagaaaatccgcgcgctggcaacagagatgcgtcagttgggtgaatctggtcagggtgcgtcccagcgcttcctcgaagcggacgtcaccttccacgagctcatcttgcgttattgccacaatgagatgttcgctgcactgattccgtcgattagcgcggttcttgtcggccgcaccgagctcggcctgcagcctgatctgccggcgcacgaggcgctagacaaccacgataagcttgccgacgccctccttaaccgcgacgccgacgccgcagaaactgcgtcccgaaacatcctcaatgaggtgcgcagcgcgctgggcacgctgaactaa

SEQ ID NO: 35 - DNA, 753 bp, synthetic construct
  misc_feature 1..753: note = gluconate repressor variant
  source 1..753: mol_type = other DNA
atgcccccagcaaacgaaagtcctatgactaatccattaggttctgcccccaccccagccaagccacttcttgacagtgttcttgatgagctcggtcaagatatcatcagtggcaaggttgctgtcggagataccttcaagctgatggacatcggcgagcgttttggtatttcccgcacagtggcacgcgaagcaatgcgcgctttggagcagctcggtcttgtcgcttcttcagctcgcattggcattactgttttgccacaggaagagtgggctgtttttgataagtccatcattcgctggcgtctcaatgacgaaggtcagcgtgaaggccagcttcagtctcttaccgagcttcgtattgctattgaaccgattgccgcgcgcagcgttgctcttcacgcgtcaaccgccgagctcgagaaaatccgcgcgctggcaacagagatgcgtcagttgggtgaatctggtcagggtgcgtcccagcgcttcctcgaagcggacgtcaccttccacgagctcatcttgcgttattgccacaatgagatgttcgctgcactgattccgtcgattagcgcggttcttgtcggccgcaccgagctcggcctgcagcctgatctgccggcgcacgaggcgctagacaaccacgataagcttgccgacgccctccttaaccgcgacgccgacgccgcagaaactgcgtcccgaaacatcctcaatgaggtgcgcagcgcgctgggcacgctgaactaa

SEQ ID NO: 36 - DNA, 753 bp, synthetic construct
  misc_feature 1..753: note = gluconate repressor variant
  source 1..753: mol_type = other DNA
atgcccccagcaaacgaaagtcctatgactaatccattaggttctgcccccaccccagccaagccacttcttgacagtgttcttgatgagctcggtcaagatatcatcagtggcaaggttgctgtcggagataccttcaagctgatggacatcggcgagcgttttggtatttcccgcacagtggcacgcgaagcaatgcgcgctttggagcagctcggtcttgtcgcttcttcacgtcgcattggcattactgttttgccacaggaagagtggcttgtttttgataagtccatcattcgctggcgtctcaatgacgaaggtcagcgtgaaggccagcttcagtctcttaccgagcttcgtattgctattgaaccgattgccgcgcgcagcgttgctcttcacgcgtcaaccgccgagctcgagaaaatccgcgcgctggcaacagagatgcgtcagttgggtgaatctggtcagggtgcgtcccagcgcttcctcgaagcggacgtcaccttccacgagctcatcttgcgttattgccacaatgagatgttcgctgcactgattccgtcgattagcgcggttcttgtcggccgcaccgagctcggcctgcagcctgatctgccggcgcacgaggcgctagacaaccacgataagcttgccgacgccctccttaaccgcgacgccgacgccgcagaaactgcgtcccgaaacatcctcaatgaggtgcgcagcgcgctgggcacgctgaactaa